European Patent Application EP 4 464 717 A1, published November 20, 2024. Title: Variants of L-threonine efflux protein and L-threonine production method using the same. Applicant: CJ CheilJedang Corporation. The sequence listing filed with the application follows.

SEQUENCE LISTING (23 sequences)

SEQ ID NO: 1 - protein, 206 aa, Escherichia coli
  REGION 1..206: note = rhtC(WT) AA
MLMLFLTVAMVHIVALMSPGPDFFFVSQTAVSRSRKEAMMGVLGITCGVMVWAGIALLGLHLIIEKMAWLHTLIMVGGGLYLCWMGYQMLRGALKKEAVSAPAPQVELAKSGRSFLKGLLTNLANPKAIIYFGSVFSLFVGDNVGTTARWGIFALIIVETLAWFTVVASLFALPQMRRGYQRLAKWIDGFAGALFAGFGIHLIISR

SEQ ID NO: 2 - DNA, 621 bp, Escherichia coli
  misc_feature 1..621: note = rhtC(WT) NT
  source 1..621: mol_type = genomic DNA
atgttgatgttatttctcaccgtcgccatggtgcacattgtggcgcttatgagccccggtcccgatttcttttttgtctctcagaccgctgtcagtcgttcccgtaaagaagcgatgatgggcgtgctgggcattacctgcggcgtaatggtttgggctgggattgcgctgcttggcctgcatttgattatcgaaaaaatggcctggctgcatacgctgattatggtgggcggtggcctgtatctctgctggatgggttaccagatgctacgtggtgcactgaaaaaagaggcggtttctgcacctgcgccacaggtcgagctggcgaaaagtgggcgcagtttcctgaaaggtttactgaccaatctcgctaatccgaaagcgattatctactttggctcggtgttctcattgtttgtcggtgataacgttggcactaccgcgcgctggggcatttttgcgctgatcattgtcgaaacgctggcgtggtttaccgtcgttgccagcctgtttgccctgccgcaaatgcgccgtggttatcaacgtctggcgaagtggattgatggttttgccggggcgttatttgccggatttggcattcatttgattatttcgcggtga

SEQ ID NO: 3 - protein, 206 aa, synthetic construct
  REGION 1..206: note = rhtC(N143I) AA
MLMLFLTVAMVHIVALMSPGPDFFFVSQTAVSRSRKEAMMGVLGITCGVMVWAGIALLGLHLIIEKMAWLHTLIMVGGGLYLCWMGYQMLRGALKKEAVSAPAPQVELAKSGRSFLKGLLTNLANPKAIIYFSSVFSLFVGDIVGTTARWGIFALIIVETLAWFTVVASLFALPQMRRGYQRLAKWIDGFAGALFAGFGIHLIISR

SEQ ID NO: 4 - DNA, 621 bp, synthetic construct
  misc_feature 1..621: note = rhtC(N143I) NT_ATT
  source 1..621: mol_type = other DNA
atgttgatgttatttctcaccgtcgccatggtgcacattgtggcgcttatgagccccggtcccgatttcttttttgtctctcagaccgctgtcagtcgttcccgtaaagaagcgatgatgggcgtgctgggcattacctgcggcgtaatggtttgggctgggattgcgctgcttggcctgcatttgattatcgaaaaaatggcctggctgcatacgctgattatggtgggcggtggcctgtatctctgctggatgggttaccagatgctacgtggtgcactgaaaaaagaggcggtttctgcacctgcgccacaggtcgagctggcgaaaagtgggcgcagtttcctgaaaggtttactgaccaatctcgctaatccgaaagcgattatctactttggctcggtgttctcattgtttgtcggtgatattgttggcactaccgcgcgctggggcatttttgcgctgatcattgtcgaaacgctggcgtggtttaccgtcgttgccagcctgtttgccctgccgcaaatgcgccgtggttatcaacgtctggcgaagtggattgatggttttgccggggcgttatttgccggatttggcattcatttgattatttcgcggtga

SEQ ID NO: 5 - DNA, 621 bp, synthetic construct
  misc_feature 1..621: note = rhtC(N143I) NT_ATC
  source 1..621: mol_type = other DNA
atgttgatgttatttctcaccgtcgccatggtgcacattgtggcgcttatgagccccggtcccgatttcttttttgtctctcagaccgctgtcagtcgttcccgtaaagaagcgatgatgggcgtgctgggcattacctgcggcgtaatggtttgggctgggattgcgctgcttggcctgcatttgattatcgaaaaaatggcctggctgcatacgctgattatggtgggcggtggcctgtatctctgctggatgggttaccagatgctacgtggtgcactgaaaaaagaggcggtttctgcacctgcgccacaggtcgagctggcgaaaagtgggcgcagtttcctgaaaggtttactgaccaatctcgctaatccgaaagcgattatctactttggctcggtgttctcattgtttgtcggtgatatcgttggcactaccgcgcgctggggcatttttgcgctgatcattgtcgaaacgctggcgtggtttaccgtcgttgccagcctgtttgccctgccgcaaatgcgccgtggttatcaacgtctggcgaagtggattgatggttttgccggggcgttatttgccggatttggcattcatttgattatttcgcggtga

SEQ ID NO: 6 - DNA, 500 bp, synthetic construct
  misc_feature 1..500: note = PrhtC
  source 1..500: mol_type = other DNA
gccatgaacattgggtgagcgtgatccgccagctgattcacctcggcctggtgacgcaaaatattgcccagcattctgccctacaactgacagaggccgcgcgcccggtgctgcgcggcgaatcctctttgcaacttgccgtgccgcgtatcgtggcgctcaaaccgaaagcgatgcagaaatcgttcggcggcaactatgatcgcaaactgttcgccaaattacgcaaactgcgtaaatcgatagccgatgaaagtaatgtcccgccgtacgtggtgtttaacgacgcaaccttgattgagatggctgaacagatgccgatcaccgccagcgaaatgctcagcgttaacggcgttgggatgcgcaagctggaacgctttggcaaaccgtttatggcgctgattcgtgcgcatgttgatggcgatgacgaagagtagtcagcagcataaaaaagtgccagtatgaagactccgtaaacgtttcccccgcgagtcaaatgt

SEQ ID NO: 7 - DNA, 40 bp, synthetic construct
  misc_feature 1..40: note = PrhtC F
  source 1..40: mol_type = other DNA
tcgagctcggtacccggggagccatgaacattgggtgagc

SEQ ID NO: 8 - DNA, 40 bp, synthetic construct
  misc_feature 1..40: note = PrhtC R
  source 1..40: mol_type = other DNA
gtcgactctagaggaggatccacatttgactcgcggggga

SEQ ID NO: 9 - DNA, 44 bp, synthetic construct
  misc_feature 1..44: note = rhtC F
  source 1..44: mol_type = other DNA
tcccccgcgagtcaaatgtgatgttgatgttatttctcaccgtc

SEQ ID NO: 10 - DNA, 45 bp, synthetic construct
  misc_feature 1..45: note = rhtC R
  source 1..45: mol_type = other DNA
gtcgactctagaggaggatctcaccgcgaaataatcaaatgaatg

SEQ ID NO: 11 - DNA, 40 bp, synthetic construct
  misc_feature 1..40: note = 1762A F
  source 1..40: mol_type = other DNA
tgaattcgagctcggtacccgtggccagtattaatgggct

SEQ ID NO: 12 - DNA, 40 bp, synthetic construct
  misc_feature 1..40: note = 1762A R
  source 1..40: mol_type = other DNA
gtctcaagcagagactcgagcaccctcaatgggtcaggcc

SEQ ID NO: 13 - DNA, 40 bp, synthetic construct
  misc_feature 1..40: note = 1762B F
  source 1..40: mol_type = other DNA
acccattgagggtgctcgagtctctgcttgagacttaagc

SEQ ID NO: 14 - DNA, 40 bp, synthetic construct
  misc_feature 1..40: note = 1762B R
  source 1..40: mol_type = other DNA
gtcgactctagaggatccccaggctctctatgggcacctc

SEQ ID NO: 15 - DNA, 40 bp, synthetic construct
  misc_feature 1..40: note = rhtC(m) F
  source 1..40: mol_type = other DNA
gcctgacccattgagggtgcgccatgaacattgggtgagc

SEQ ID NO: 16 - DNA, 50 bp, synthetic construct
  misc_feature 1..50: note = rhtC(m) R
  source 1..50: mol_type = other DNA
ataacgcttaagtctcaagcagagactcgatcaccgcgaaataatcaaat

SEQ ID NO: 17 - DNA, 22 bp, synthetic construct
  misc_feature 1..22: note = pDC F
  source 1..22: mol_type = other DNA
ctattacgccagctggcgaaag

SEQ ID NO: 18 - DNA, 20 bp, synthetic construct
  misc_feature 1..20: note = pDC R
  source 1..20: mol_type = other DNA
atgttgtgtggaattgtgag

SEQ ID NO: 19 - DNA, 20 bp, synthetic construct
  misc_feature 1..20: note = seq 1
  source 1..20: mol_type = other DNA
ttctcttgttcctttctgag

SEQ ID NO: 20 - DNA, 20 bp, synthetic construct
  misc_feature 1..20: note = seq 2
  source 1..20: mol_type = other DNA
ttctgagtagctgagcttcg

SEQ ID NO: 21 - DNA, 20 bp, synthetic construct
  misc_feature 1..20: note = seq 3
  source 1..20: mol_type = other DNA
ccagatgctacgtggtgcac

SEQ ID NO: 22 - DNA, 20 bp, synthetic construct
  misc_feature 1..20: note = seq 4
  source 1..20: mol_type = other DNA
tggtctgctcgcttctcgat

SEQ ID NO: 23 - DNA, 20 bp, synthetic construct
  misc_feature 1..20: note = seq 5
  source 1..20: mol_type = other DNA
tatcttcgtagagcactgct